European Patent Specification EP 3 212 225 B1, published November 19, 2025. Title: METHODS AND COMPOSITIONS FOR MODIFIED T CELLS. Applicant: University of Pennsylvania Zhao, Yangbing Liu, Xiaojun June, Carl. The sequence listing filed with the application follows.

SEQUENCE LISTING (52 sequences)

SEQ ID NO: 1 - protein, 58 aa, Artificial Sequence
  affinity antibody mimetic
VDNKFNKELEKAYNEIRNLPNLNGWQMTAFIASLVDDPSQSANLLAEAKKLNDAQAPK

SEQ ID NO: 2 - protein, 58 aa, Artificial Sequence
  affinity antibody mimetic
VDNKFNKEMLIAMEEIGSLPNLNWGQEQAFILSLWDDPSQSANLLAEAKKLNDAQAPK

SEQ ID NO: 3 - protein, 58 aa, Artificial Sequence
  affinity antibody mimetic
VDNKFNKEFWWASDEIRNLPNLNGWQMTAFIASLADDPSQSANLLAEAKKLNDAQAPK

SEQ ID NO: 4 - protein, 58 aa, Artificial Sequence
  affinity antibody mimetic
VDNKFNKEMWAAWEEIRNLPNLNGWQMTAFIASLVDDPSQSANLLAEAKKLNDAQAPK

SEQ ID NO: 5 - protein, 58 aa, Artificial Sequence
  affinity antibody mimetic
VDNKFNKEMRNAYWEIALLPNLNNQQKRAFIRSLYDDPSQSANLLAEAKKLNDAQAPK

SEQ ID NO: 6 - protein, 58 aa, Artificial Sequence
  affinity antibody mimetic
VDNKFNKEMRNAYWEIALLPNLTNQQKRAFIRSLYKDPSQSANLLAEAKKLNDAQAPK

SEQ ID NO: 7 - protein, 58 aa, Artificial Sequence
  affinity antibody mimetic
VDNKFNKEMRNAYWEIALLPNLNNQQKRAFIRSLYADPSQSANLLAEAKKLNDAQAPK

SEQ ID NO: 8 - protein, 58 aa, Artificial Sequence
  affinity antibody mimetic
VDNKFEKEMRNAYWEIALLPNLTNQQKRAFIRSLYDDPSQSANLLAEAKKLNDAQAPK

SEQ ID NO: 9 - DNA, 243 bp, Artificial Sequence
  affinity antibody mimetic
atggcgctgcccgtgacggccctgctgctccccctggcactgcttctgcacgccgcccgaccctctcaggtcgacaacaagtttaacaaggaattggagaaggcgtacaacgaaatccggaacctgcccaacctcaacggatggcagatgactgctttcatcgcgtccctggtggacgacccctcccagtcggcgaacctgctggccgaggccaagaaactgaatgacgcccaagcccctaag

SEQ ID NO: 10 - DNA, 243 bp, Artificial Sequence
  affinity antibody mimetic
atggcgctgcccgtgacggccctactcctgccactggcactcctgctccacgccgcgcggccatcccaggtggacaacaaattcaacaaggagatgctcatcgcaatggaagaaataggctccctccccaacctgaactgggggcaggagcaggcgttcatactctcgctctgggatgacccaagccagtctgcgaacctccttgccgaggcgaagaagctcaatgacgctcaggcacccaag

SEQ ID NO: 11 - DNA, 243 bp, Artificial Sequence
  affinity antibody mimetic
atggcgctgcccgtgacggccctcttgctgcccctggccctcctgctccacgcagccaggccgagtcaagtcgacaacaagtttaacaaggaattctggtgggcctccgacgagatccgcaatctgcccaacctgaacggctggcagatgaccgccttcatcgcaagcctggcggacgacccttcccagagtgccaacctgctggcagaggccaagaagctgaacgacgcccaagcgccaaag

SEQ ID NO: 12 - DNA, 270 bp, Artificial Sequence
  affinity antibody mimetic
atggcgctgcccgtgacggccctgctgctgccgctcgccttactgctccacgcggctaggccctcccaggtggataacaagttcaacaaggagatgtgggccgcctgggaggaaatccgcaacctcccaaatctgaacggctggcagatgacagcattcattgcctccctggtggacgatccatcgcagtcggccaacctcctagccgaggccaagaagctgaacgacgcccaggcgcccaagcatcatcaccatcatcataccacgacg

SEQ ID NO: 13 - DNA, 243 bp, Artificial Sequence
  affinity antibody mimetic
atggcgctgcccgtgacggcccttctgctcccgctggccctgctgctgcatgccgcccgcccctcacaagtcgacaacaaattcaataaggagatgagaaacgcttactgggagatcgccctgcttcccaacctgaacaaccagcagaaacgagcattcattcgcagcctctacgacgatccgtcgcagtcagctaatctcctcgccgaggcgaagaagctgaacgacgcccaggcccccaag

SEQ ID NO: 14 - DNA, 243 bp, Artificial Sequence
  affinity antibody mimetic
atggcgctgcccgtgacggccctcctgctgcccctggccctgctgctccacgctgcaagacccagccaggtggacaacaagtttaacaaggagatgcgcaacgcctactgggagatcgccctcctgcccaacttaaccaaccagcaaaaaagagctttcattcgttccctgtacaaagacccttcgcagtccgccaatctgcttgccgaggctaagaagctgaacgacgcgcaggcccccaag

SEQ ID NO: 15 - DNA, 243 bp, Artificial Sequence
  affinity antibody mimetic
atggcgctgcccgtgacggccctcctgctgcccctcgcgctcctgctccacgccgcccggccctcccaagtcgacaacaagttcaataaggagatgcggaacgcatactgggagatcgccctgctgccgaacctgaacaaccagcagaagcgtgcctttatcaggtctctctacgcagatccaagccagtctgcgaacctgctggccgaggcgaagaaactcaacgacgcgcaggcaccgaag

SEQ ID NO: 16 - DNA, 243 bp, Artificial Sequence
  affinity antibody mimetic
atggcgctgcccgtgacggccctgctcctgccgctcgccctcttacttcacgccgcgcgaccgtcccaggttgacaacaagttcgagaaagagatgaggaacgcatactgggagatcgccttactgcctaatctgactaaccagcagaagcgcgccttcatccgctccctgtacgacgatccgtcgcagtccgctaacttgctggccgaggccaagaagctcaacgatgcccaagcccccaag

SEQ ID NO: 17 - DNA, 18 bp, Artificial Sequence
  affinity antibody mimetic
catcatcaccatcatcat

SEQ ID NO: 18 - DNA, 672 bp, Artificial Sequence
  affinity antibody mimetic
accacgacgccagcgccgcgaccaccaacaccggcgcccaccatcgcgtcgcagcccctgtccctgcgcccagaggcgtgccggccagcggcggggggcgcagtgcacacgagggggctggacttcgcctgtgatatctacatctgggcgcccttggccgggacttgtggggtccttctcctgtcactggttatcaccctttactgcaaacggggcagaaagaaactcctgtatatattcaaacaaccatttatgagaccagtacaaactactcaagaggaagatggctgtagctgccgatttccagaagaagaagaaggaggatgtgaactgagagtgaagttcagcaggagcgcagacgcccccgcgtacaagcagggccagaaccagctctataacgagctcaatctaggacgaagagaggagtacgacgttttggacaagagacgtggccgggaccctgagatggggggaaagccgagaaggaagaaccctcaggaaggcctgtacaatgaactgcagaaagataagatggcggaggcctacagtgagattgggatgaaaggcgagcgccggaggggcaaggggcacgatggcctttaccagggtctcagtacagccaccaaggacacctacgacgcccttcacatgcaggccctgccccctcgctaa

SEQ ID NO: 19 - DNA, 774 bp, Artificial Sequence
  affinity antibody mimetic
ggaggtggtggatccgatatcaaactgcagcagtcaggggctgaactggcaagacctggggcctcagtgaagatgtcctgcaagacttctggctacacctttactaggtacacgatgcactgggtaaaacagaggcctggacagggtctggaatggattggatacattaatcctagccgtggttatactaattacaatcagaagttcaaggacaaggccacattgactacagacaaatcctccagcacagcctacatgcaactgagcagcctgacatctgaggactctgcggtctatttctgtgcaagatattatgatgatcattactgccttgactactggggccaaggcaccactctcacagtctcctcagtcgaaggtggaagtggaggttctggtggaagtggaggttcaggtggagtcgacgacgccgccattcagctgacccagtctccagcaatcatgtctgcatctccaggggagaaggtcaccatgacctgcagagccagttcaagtgtaagttacatgaactggtaccagcagaagtcaggcacctcccccaaaagatggatttatgacacatccaaagtggcttctggagtcccttatcgcttcagtggcagtgggtctgggacctcatactctctcacaatcagcagcatggaggctgaagatgctgccacttattactgccaacagtggagtagtaacccgctcacgttcggtgctgggaccaagctggagctgaaacatcatcaccatcatcattaataa

SEQ ID NO: 20 - DNA, 1500 bp, Artificial Sequence
  affinity antibody mimetic
atgggctggtcttgcatcatcctgtttctggtcgccaccgccaccggggtccacagtgagatcgttctcacccaatcccccgccacactgtcgctctccccaggcgagcgggccacgctgtcgtgtcgcgcgagccagagcgtttcctcctacctcgcctggtaccagcagaagccgggccaggcccctcgcctgctgatctacgatacttcgaatagagccaccggtatccctgcaaggttctccggatccgggtcagggacggatttcaccctgaccatttcctccctggagccagaggatttcgccgtgtactactgccagcagcgcagtaactggcctctgactttcggtggcggcacaaaggtggagatcaaggggggcggcggcagtgggggcgggggcagcgggggcggaggctcgcaggtccagctcgtggagtcggggggggacgtggtccagccaggcaggagcctgaggctgtcatgcgctgcgtccggcctgacgttcaccaactacggcttccactgggtgagacaggcacccgggaagggcctggaatgggtggccgtgatctggtacgacgggagcaagaagtactacgcagactcagtgaagggccgattcaccatcagccgggacaactctaagaacacactgtacctgcagatgaacaatttgcgcgccgaggataccgccgtatattattgcgccacaggcgacgactattggggacagggcaccctggtcacggtaagtagtggaggtggtggatcccaggtacaactgcagcagtctgggcctgagctggagaagcctggcgcttcagtgaagatatcctgcaaggcttctggttactcattcactggctacaccatgaactgggtgaagcagagccatggaaagagccttgagtggattggacttattactccttacaatggtgcttctagctacaaccagaagttcaggggcaaggccacattaactgtagacaagtcatccagcacagcctacatggacctcctcagtctgacatctgaagactctgcagtctatttctgtgcaagggggggttacgacgggaggggttttgactactggggccaagggaccacggtcaccgtctcctcaggtggaggcggttcaggcggcggtggctctagcggtggcggatcggacatcgagctcactcagtctccagcaatcatgtctgcatctccaggggagaaggtcaccatgacctgcagtgccagctcaagtgtaagttacatgcactggtaccagcagaagtcaggcacctcccccaaaagatggatttacgacacatccaaactggcttctggagtcccaggtcgcttcagtggcagtgggtctggaaactcttactctctcacaatcagcagcgtggaggctgaagacgacgcaacttattactgccagcagtggagtaagcaccctctcacgtacggtgctgggacaaagttggaaatcaaataa

SEQ ID NO: 21 - DNA, 1524 bp, Artificial Sequence
  affinity antibody mimetic
atgggctggtcctgtatcatattattcctggtcgcgaccgccaccggggtgcactccgacatccagatgactcagtccccatcctccctgtcggcgtccgttggcgaccgggtctcgattacatgccgcgcctcccagggcatctcctcctggctcgcctggtaccagcagaagcctgagaaggcccccaagtcattaatctacgcagcctccaatctgaggtccggcgtgcccagtagattctcgggctccgggtcgggcactgattttaccctcaccatcagttcgctccagccagaggacttcgctacgtactattgccagcagtactattcctacccacgcaccttcgggcagggcaccaaggtcgagatcaagggcggcggcgggtccggcggaggcgggtctggcggtggtggttcgcagctgcagctgcaagagtccgggcctggcctcgtgaagcccagcgagaccctgtcattgacatgcaccgtgagtggggggagtctgtcccgctcctccttcttctggggctggattcgccagccgcccggcaaggggctggaatggatcgggtcgatctactacagtgggtcgacttactacaatccaagtctgaagagccgtgtgaccatctcagtggatacctcgaagaatcagttcagcctgaagctctcctccgtcaccgcggccgatacggcagtgtactactgtgtgcgcgattacgacatcctcactggcgatgaggactactggggtcaaggcaccctagtcacggtgtcgtcgggaggtggtggatcccaggtacaactgcagcagtctgggcctgagctggagaagcctggcgcttcagtgaagatatcctgcaaggcttctggttactcattcactggctacaccatgaactgggtgaagcagagccatggaaagagccttgagtggattggacttattactccttacaatggtgcttctagctacaaccagaagttcaggggcaaggccacattaactgtagacaagtcatccagcacagcctacatggacctcctcagtctgacatctgaagactctgcagtctatttctgtgcaagggggggttacgacgggaggggttttgactactggggccaagggaccacggtcaccgtctcctcaggtggaggcggttcaggcggcggtggctctagcggtggcggatcggacatcgagctcactcagtctccagcaatcatgtctgcatctccaggggagaaggtcaccatgacctgcagtgccagctcaagtgtaagttacatgcactggtaccagcagaagtcaggcacctcccccaaaagatggatttacgacacatccaaactggcttctggagtcccaggtcgcttcagtggcagtgggtctggaaactcttactctctcacaatcagcagcgtggaggctgaagacgacgcaacttattactgccagcagtggagtaagcaccctctcacgtacggtgctgggacaaagttggaaatcaaataa

SEQ ID NO: 22 - DNA, 1500 bp, Artificial Sequence
  affinity antibody mimetic
atggggtggagttgcatcattctgttcctcgtggcgaccgcaacaggcgtgcacagcgagatcgtgctcacccagtcaccagccaccttatccttaagtcccggcgaacgcgccaccctgtcctgcagagcgtcccagtcggtcagcagttatctggcgtggtaccagcagaagcccggccaagccccacgcctgctcatctacgacgcgtcgaatcgcgccacgggtattcccgcacggtttagcggctccggttcagggactgactttaccctgacgatctcgagtctagagccggaggacttcgcggtgtactactgccagcagtccagcaactggccgcgcaccttcggccagggcacaaaggtggagatcaaggggggcgggggctcgggtggcgggggctccggaggcgggggctcccaagtgtacctggttgaatcgggcgggggcgtggtgcagcctgggcgctcgctgcgcctcagttgcgccgcgtccggattcacattttccaactacgggatgcactgggtgcgccaagctccgggaaaggggctggagtgggtggccctgatctggtacgacggttccaataagtactatgccgatagcgtgaagggccggttcacgatatccagggataactccaagaacactctctatctgcagatgacctcactgcgcgtggaggacactgccgtctattactgcgcctccaatgtggatcactggggacagggcaccctggtgaccgtaagctcgggaggtggtggatcccaggtacaactgcagcagtctgggcctgagctggagaagcctggcgcttcagtgaagatatcctgcaaggcttctggttactcattcactggctacaccatgaactgggtgaagcagagccatggaaagagccttgagtggattggacttattactccttacaatggtgcttctagctacaaccagaagttcaggggcaaggccacattaactgtagacaagtcatccagcacagcctacatggacctcctcagtctgacatctgaagactctgcagtctatttctgtgcaagggggggttacgacgggaggggttttgactactggggccaagggaccacggtcaccgtctcctcaggtggaggcggttcaggcggcggtggctctagcggtggcggatcggacatcgagctcactcagtctccagcaatcatgtctgcatctccaggggagaaggtcaccatgacctgcagtgccagctcaagtgtaagttacatgcactggtaccagcagaagtcaggcacctcccccaaaagatggatttacgacacatccaaactggcttctggagtcccaggtcgcttcagtggcagtgggtctggaaactcttactctctcacaatcagcagcgtggaggctgaagacgacgcaacttattactgccagcagtggagtaagcaccctctcacgtacggtgctgggacaaagttggaaatcaaataa

SEQ ID NO: 23 - DNA, 1434 bp, Artificial Sequence
  affinity antibody mimetic
atgggctggtcttgcatcatcctgtttctggtcgccaccgccaccggggtccacagtgagatcgttctcacccaatcccccgccacactgtcgctctccccaggcgagcgggccacgctgtcgtgtcgcgcgagccagagcgtttcctcctacctcgcctggtaccagcagaagccgggccaggcccctcgcctgctgatctacgatacttcgaatagagccaccggtatccctgcaaggttctccggatccgggtcagggacggatttcaccctgaccatttcctccctggagccagaggatttcgccgtgtactactgccagcagcgcagtaactggcctctgactttcggtggcggcacaaaggtggagatcaaggggggcggcggcagtgggggcgggggcagcgggggcggaggctcgcaggtccagctcgtggagtcggggggggacgtggtccagccaggcaggagcctgaggctgtcatgcgctgcgtccggcctgacgttcaccaactacggcttccactgggtgagacaggcacccgggaagggcctggaatgggtggccgtgatctggtacgacgggagcaagaagtactacgcagactcagtgaagggccgattcaccatcagccgggacaactctaagaacacactgtacctgcagatgaacaatttgcgcgccgaggataccgccgtatattattgcgccacaggcgacgactattggggacagggcaccctggtcacggtaagtagtaccacgacgccagcgccgcgaccaccaacaccggcgcccaccatcgcgtcgcagcccctgtccctgcgcccagaggcgtgccggccagcggcggggggcgcagtgcacacgagggggctggacttcgcctgtgatatctacatctgggcgcccttggccgggacttgtggggtccttctcctgtcactggttatcaccctttactgcaaacggggcagaaagaaactcctgtatatattcaaacaaccatttatgagaccagtacaaactactcaagaggaagatggctgtagctgccgatttccagaagaagaagaaggaggatgtgaactgagagtgaagttcagcaggagcgcagacgcccccgcgtacaagcagggccagaaccagctctataacgagctcaatctaggacgaagagaggagtacgacgttttggacaagagacgtggccgggaccctgagatggggggaaagccgagaaggaagaaccctcaggaaggcctgtacaatgaactgcagaaagataagatggcggaggcctacagtgagattgggatgaaaggcgagcgccggaggggcaaggggcacgatggcctttaccagggtctcagtacagccaccaaggacacctacgacgcccttcacatgcaggccctgccccctcgctaa

SEQ ID NO: 24 - DNA, 1458 bp, Artificial Sequence
  affinity antibody mimetic
atgggctggtcctgtatcatattattcctggtcgcgaccgccaccggggtgcactccgacatccagatgactcagtccccatcctccctgtcggcgtccgttggcgaccgggtctcgattacatgccgcgcctcccagggcatctcctcctggctcgcctggtaccagcagaagcctgagaaggcccccaagtcattaatctacgcagcctccaatctgaggtccggcgtgcccagtagattctcgggctccgggtcgggcactgattttaccctcaccatcagttcgctccagccagaggacttcgctacgtactattgccagcagtactattcctacccacgcaccttcgggcagggcaccaaggtcgagatcaagggcggcggcgggtccggcggaggcgggtctggcggtggtggttcgcagctgcagctgcaagagtccgggcctggcctcgtgaagcccagcgagaccctgtcattgacatgcaccgtgagtggggggagtctgtcccgctcctccttcttctggggctggattcgccagccgcccggcaaggggctggaatggatcgggtcgatctactacagtgggtcgacttactacaatccaagtctgaagagccgtgtgaccatctcagtggatacctcgaagaatcagttcagcctgaagctctcctccgtcaccgcggccgatacggcagtgtactactgtgtgcgcgattacgacatcctcactggcgatgaggactactggggtcaaggcaccctagtcacggtgtcgtcgaccacgacgccagcgccgcgaccaccaacaccggcgcccaccatcgcgtcgcagcccctgtccctgcgcccagaggcgtgccggccagcggcggggggcgcagtgcacacgagggggctggacttcgcctgtgatatctacatctgggcgcccttggccgggacttgtggggtccttctcctgtcactggttatcaccctttactgcaaacggggcagaaagaaactcctgtatatattcaaacaaccatttatgagaccagtacaaactactcaagaggaagatggctgtagctgccgatttccagaagaagaagaaggaggatgtgaactgagagtgaagttcagcaggagcgcagacgcccccgcgtacaagcagggccagaaccagctctataacgagctcaatctaggacgaagagaggagtacgacgttttggacaagagacgtggccgggaccctgagatggggggaaagccgagaaggaagaaccctcaggaaggcctgtacaatgaactgcagaaagataagatggcggaggcctacagtgagattgggatgaaaggcgagcgccggaggggcaaggggcacgatggcctttaccagggtctcagtacagccaccaaggacacctacgacgcccttcacatgcaggccctgccccctcgctaa

SEQ ID NO: 25 - DNA, 1434 bp, Artificial Sequence
  affinity antibody mimetic
atggggtggagttgcatcattctgttcctcgtggcgaccgcaacaggcgtgcacagcgagatcgtgctcacccagtcaccagccaccttatccttaagtcccggcgaacgcgccaccctgtcctgcagagcgtcccagtcggtcagcagttatctggcgtggtaccagcagaagcccggccaagccccacgcctgctcatctacgacgcgtcgaatcgcgccacgggtattcccgcacggtttagcggctccggttcagggactgactttaccctgacgatctcgagtctagagccggaggacttcgcggtgtactactgccagcagtccagcaactggccgcgcaccttcggccagggcacaaaggtggagatcaaggggggcgggggctcgggtggcgggggctccggaggcgggggctcccaagtgtacctggttgaatcgggcgggggcgtggtgcagcctgggcgctcgctgcgcctcagttgcgccgcgtccggattcacattttccaactacgggatgcactgggtgcgccaagctccgggaaaggggctggagtgggtggccctgatctggtacgacggttccaataagtactatgccgatagcgtgaagggccggttcacgatatccagggataactccaagaacactctctatctgcagatgacctcactgcgcgtggaggacactgccgtctattactgcgcctccaatgtggatcactggggacagggcaccctggtgaccgtaagctcgaccacgacgccagcgccgcgaccaccaacaccggcgcccaccatcgcgtcgcagcccctgtccctgcgcccagaggcgtgccggccagcggcggggggcgcagtgcacacgagggggctggacttcgcctgtgatatctacatctgggcgcccttggccgggacttgtggggtccttctcctgtcactggttatcaccctttactgcaaacggggcagaaagaaactcctgtatatattcaaacaaccatttatgagaccagtacaaactactcaagaggaagatggctgtagctgccgatttccagaagaagaagaaggaggatgtgaactgagagtgaagttcagcaggagcgcagacgcccccgcgtacaagcagggccagaaccagctctataacgagctcaatctaggacgaagagaggagtacgacgttttggacaagagacgtggccgggaccctgagatggggggaaagccgagaaggaagaaccctcaggaaggcctgtacaatgaactgcagaaagataagatggcggaggcctacagtgagattgggatgaaaggcgagcgccggaggggcaaggggcacgatggcctttaccagggtctcagtacagccaccaaggacacctacgacgcccttcacatgcaggccctgccccctcgctaa

SEQ ID NO: 26 - DNA, 714 bp, Artificial Sequence
  affinity antibody mimetic
atgcagatcccacaggcgccctggccagtcgtctgggcggtgctacaactgggctggcggccaggatggttcttagactccccagacaggccctggaacccccccaccttctccccagccctgctcgtggtgaccgaaggggacaacgccaccttcacctgcagcttctccaacacatcggagagcttcgtgctaaactggtaccgcatgagccccagcaaccagacggacaagctggccgccttccccgaggaccgcagccagcccggccaggactgccgcttccgtgtcacacaactgcccaacgggcgtgacttccacatgagcgtggtcagggcccggcgcaatgacagcggcacctacctctgtggggccatctccctggcccccaaggcgcagatcaaagagagcctgcgggcagagctcagggtgacagagagaagggcagaagtgcccacagcccaccccagcccctcacccaggccagccggccagttccaaaccctggtgttttgggtgctggtggtggttggtggagtcctggcttgctatagcttgctagtaacagtggcctttattattttctgggtgaggagtaagaggagcaggctcctgcacagtgacttcttcttctttactgcccgccgcgccgggcccacccgcaagcattaccaggcctatgccgcaccacgcgacttcgcagcctatcgctcc

SEQ ID NO: 27 - DNA, 933 bp, Artificial Sequence
  affinity antibody mimetic
atgcagatcccacaggcgccctggccagtcgtctgggcggtgctacaactgggctggcggccaggatggttcttagactccccagacaggccctggaacccccccaccttctccccagccctgctcgtggtgaccgaaggggacaacgccaccttcacctgcagcttctccaacacatcggagagcttcgtgctaaactggtaccgcatgagccccagcaaccagacggacaagctggccgccttccccgaggaccgcagccagcccggccaggactgccgcttccgtgtcacacaactgcccaacgggcgtgacttccacatgagcgtggtcagggcccggcgcaatgacagcggcacctacctctgtggggccatctccctggcccccaaggcgcagatcaaagagagcctgcgggcagagctcagggtgacagagagaagggcagaagtgcccacagcccaccccagcccctcacccaggccagccggccagttccaaaccctggtgttttgggtgctggtggtggttggtggagtcctggcttgctatagcttgctagtaacagtggcctttattattttctgggtggatagagtgaagttcagcaggagcgcagacgcccccgcgtaccagcagggccagaaccagctctataacgagctcaatctaggacgaagagaggagtacgatgttttggacaagagacgtggccgggaccctgagatggggggaaagccgagaaggaagaaccctcaggaaggcctgtacaatgaactgcagaaagataagatggcggaggcctacagtgagattgggatgaaaggcgagcgccggaggggcaaggggcacgatggcctttaccagggtctcagtacagccaccaaggacacctacgacgcccttcacatgcaggccctgccccctcgctaa

SEQ ID NO: 28 - DNA, 1512 bp, Artificial Sequence
  affinity antibody mimetic
atgggctggtcttgcatcatcctgtttctggtcgccaccgccaccggggtccacagtgagatcgttctcacccaatcccccgccacactgtcgctctccccaggcgagcgggccacgctgtcgtgtcgcgcgagccagagcgtttcctcctacctcgcctggtaccagcagaagccgggccaggcccctcgcctgctgatctacgatacttcgaatagagccaccggtatccctgcaaggttctccggatccgggtcagggacggatttcaccctgaccatttcctccctggagccagaggatttcgccgtgtactactgccagcagcgcagtaactggcctctgactttcggtggcggcacaaaggtggagatcaaggggggcggcggcagtgggggcgggggcagcgggggcggaggctcgcaggtccagctcgtggagtcggggggggacgtggtccagccaggcaggagcctgaggctgtcatgcgctgcgtccggcctgacgttcaccaactacggcttccactgggtgagacaggcacccgggaagggcctggaatgggtggccgtgatctggtacgacgggagcaagaagtactacgcagactcagtgaagggccgattcaccatcagccgggacaactctaagaacacactgtacctgcagatgaacaatttgcgcgccgaggataccgccgtatattattgcgccacaggcgacgactattggggacagggcaccctggtcacggtaagtagtggaggtggtggatccgacatccagatgacccagtccccttcctccctctctgcctctgtgggagaccgcgttaccatcacatgccgagcttcccaggacgtgaacacagccgtggcctggtaccagcagaagcccgggaaggcacccaaactcctcatctactccgcctccttcctatacagtggcgtgccttcccgattctccggctccaggagtggcacggactttacgctcaccattagtagcctgcagcccgaagacttcgcgacctactattgtcagcaacactacacgacgccaccaactttcggccagggtaccaaggtcgagattaagcgaaccggcagtaccagtgggtctggcaagcccggcagcggcgagggatccgaggtccagctggtcgagtccggcgggggcctggtgcagccgggcggctcgctgaggttatcttgcgccgccagtggcttcaacatcaaggatacttacatccactgggtgaggcaggctccgggcaagggcctggaatgggtggctaggatctaccctactaacgggtacacacgctacgcagattcggtgaaaggccgcttcactatctccgccgacacctcgaagaacactgcttacctgcagatgaactccctcagggccgaagatactgcagtctactactgctcccgctggggtggggacggcttctacgccatggacgtgtggggtcagggcactctagttacagtgtcatcctaa

SEQ ID NO: 29 - DNA, 1536 bp, Artificial Sequence
  affinity antibody mimetic
atgggctggtcctgtatcatattattcctggtcgcgaccgccaccggggtgcactccgacatccagatgactcagtccccatcctccctgtcggcgtccgttggcgaccgggtctcgattacatgccgcgcctcccagggcatctcctcctggctcgcctggtaccagcagaagcctgagaaggcccccaagtcattaatctacgcagcctccaatctgaggtccggcgtgcccagtagattctcgggctccgggtcgggcactgattttaccctcaccatcagttcgctccagccagaggacttcgctacgtactattgccagcagtactattcctacccacgcaccttcgggcagggcaccaaggtcgagatcaagggcggcggcgggtccggcggaggcgggtctggcggtggtggttcgcagctgcagctgcaagagtccgggcctggcctcgtgaagcccagcgagaccctgtcattgacatgcaccgtgagtggggggagtctgtcccgctcctccttcttctggggctggattcgccagccgcccggcaaggggctggaatggatcgggtcgatctactacagtgggtcgacttactacaatccaagtctgaagagccgtgtgaccatctcagtggatacctcgaagaatcagttcagcctgaagctctcctccgtcaccgcggccgatacggcagtgtactactgtgtgcgcgattacgacatcctcactggcgatgaggactactggggtcaaggcaccctagtcacggtgtcgtcgggaggtggtggatccgacatccagatgacccagtccccttcctccctctctgcctctgtgggagaccgcgttaccatcacatgccgagcttcccaggacgtgaacacagccgtggcctggtaccagcagaagcccgggaaggcacccaaactcctcatctactccgcctccttcctatacagtggcgtgccttcccgattctccggctccaggagtggcacggactttacgctcaccattagtagcctgcagcccgaagacttcgcgacctactattgtcagcaacactacacgacgccaccaactttcggccagggtaccaaggtcgagattaagcgaaccggcagtaccagtgggtctggcaagcccggcagcggcgagggatccgaggtccagctggtcgagtccggcgggggcctggtgcagccgggcggctcgctgaggttatcttgcgccgccagtggcttcaacatcaaggatacttacatccactgggtgaggcaggctccgggcaagggcctggaatgggtggctaggatctaccctactaacgggtacacacgctacgcagattcggtgaaaggccgcttcactatctccgccgacacctcgaagaacactgcttacctgcagatgaactccctcagggccgaagatactgcagtctactactgctcccgctggggtggggacggcttctacgccatggacgtgtggggtcagggcactctagttacagtgtcatcctaa

SEQ ID NO: 30 - DNA, 1512 bp, Artificial Sequence
  affinity antibody mimetic
atggggtggagttgcatcattctgttcctcgtggcgaccgcaacaggcgtgcacagcgagatcgtgctcacccagtcaccagccaccttatccttaagtcccggcgaacgcgccaccctgtcctgcagagcgtcccagtcggtcagcagttatctggcgtggtaccagcagaagcccggccaagccccacgcctgctcatctacgacgcgtcgaatcgcgccacgggtattcccgcacggtttagcggctccggttcagggactgactttaccctgacgatctcgagtctagagccggaggacttcgcggtgtactactgccagcagtccagcaactggccgcgcaccttcggccagggcacaaaggtggagatcaaggggggcgggggctcgggtggcgggggctccggaggcgggggctcccaagtgtacctggttgaatcgggcgggggcgtggtgcagcctgggcgctcgctgcgcctcagttgcgccgcgtccggattcacattttccaactacgggatgcactgggtgcgccaagctccgggaaaggggctggagtgggtggccctgatctggtacgacggttccaataagtactatgccgatagcgtgaagggccggttcacgatatccagggataactccaagaacactctctatctgcagatgacctcactgcgcgtggaggacactgccgtctattactgcgcctccaatgtggatcactggggacagggcaccctggtgaccgtaagctcgggaggtggtggatccgacatccagatgacccagtccccttcctccctctctgcctctgtgggagaccgcgttaccatcacatgccgagcttcccaggacgtgaacacagccgtggcctggtaccagcagaagcccgggaaggcacccaaactcctcatctactccgcctccttcctatacagtggcgtgccttcccgattctccggctccaggagtggcacggactttacgctcaccattagtagcctgcagcccgaagacttcgcgacctactattgtcagcaacactacacgacgccaccaactttcggccagggtaccaaggtcgagattaagcgaaccggcagtaccagtgggtctggcaagcccggcagcggcgagggatccgaggtccagctggtcgagtccggcgggggcctggtgcagccgggcggctcgctgaggttatcttgcgccgccagtggcttcaacatcaaggatacttacatccactgggtgaggcaggctccgggcaagggcctggaatgggtggctaggatctaccctactaacgggtacacacgctacgcagattcggtgaaaggccgcttcactatctccgccgacacctcgaagaacactgcttacctgcagatgaactccctcagggccgaagatactgcagtctactactgctcccgctggggtggggacggcttctacgccatggacgtgtggggtcagggcactctagttacagtgtcatcctaa

SEQ ID NO: 31 - DNA, 1505 bp, Artificial Sequence
  affinity antibody mimetic
atgggctggtcttgcatcatcctgtttctggtcgccaccgccaccggggtccacagtgagatcgttctcacccaatcccccgccacactgtcgctctccccaggcgagcgggccacgctgtcgtgtcgcgcgagccagagcgtttcctcctacctcgcctggtaccagcagaagccgggccaggcccctcgcctgctgatctacgatacttcgaatagagccaccggtatccctgcaaggttctccggatccgggtcagggacggatttcaccctgaccatttcctccctggagccagaggatttcgccgtgtactactgccagcagcgcagtaactggcctctgactttcggtggcggcacaaaggtggagatcaaggggggcggcggcagtgggggcgggggcagcgggggcggaggctcgcaggtccagctcgtggagtcggggggggacgtggtccagccaggcaggagcctgaggctgtcatgcgctgcgtccggcctgacgttcaccaactacggcttccactgggtgagacaggcacccgggaagggcctggaatgggtggccgtgatctggtacgacgggagcaagaagtactacgcagactcagtgaagggccgattcaccatcagccgggacaactctaagaacacactgtacctgcagatgaacaatttgcgcgccgaggataccgccgtatattattgcgccacaggcgacgactattggggacagggcaccctggtcacggtaagtagtggaggtggtggatccgacatccagatgacacagactacatcctccctgtctgcctctctgggagacagagtcaccatcagttgcagggcaagtcaggacattagtaaatatttaaattggtatcagcagaaaccagatggaactgttaaactcctgatctaccatacatcaagattacactcaggagtcccatcaaggttcagtggcagtgggtctggaacagattattctctcaccattagcaacctggagcaagaagatattgccacttacttttgccaacagggtaatacgcttccgtacacgttcggaggggggaccaagctggagatcacaggtggcggtggctcgggcggtggtgggtcgggtggcggcggatctgaggtgaaactgcaggagtcaggacctggcctggtggcgccctcacagagcctgtccgtcacatgcactgtctcaggggtctcattacccgactatggtgtaagctggattcgccagcctccacgaaagggtctggagtggctgggagtaatatggggtagtgaaaccacatactataattcagctctcaaatccagactgaccatcatcaaggacaactccaagagccaagttttcttaaaaatgaacagtctgcaaactgacgacacagccatttactactgtgccaaacattattactacggtggtagctacgctatggactactggggccaaggaacctcagtcaccgtctcctctaa

SEQ ID NO: 32 - DNA, 1529 bp, Artificial Sequence
  affinity antibody mimetic
atgggctggtcctgtatcatattattcctggtcgcgaccgccaccggggtgcactccgacatccagatgactcagtccccatcctccctgtcggcgtccgttggcgaccgggtctcgattacatgccgcgcctcccagggcatctcctcctggctcgcctggtaccagcagaagcctgagaaggcccccaagtcattaatctacgcagcctccaatctgaggtccggcgtgcccagtagattctcgggctccgggtcgggcactgattttaccctcaccatcagttcgctccagccagaggacttcgctacgtactattgccagcagtactattcctacccacgcaccttcgggcagggcaccaaggtcgagatcaagggcggcggcgggtccggcggaggcgggtctggcggtggtggttcgcagctgcagctgcaagagtccgggcctggcctcgtgaagcccagcgagaccctgtcattgacatgcaccgtgagtggggggagtctgtcccgctcctccttcttctggggctggattcgccagccgcccggcaaggggctggaatggatcgggtcgatctactacagtgggtcgacttactacaatccaagtctgaagagccgtgtgaccatctcagtggatacctcgaagaatcagttcagcctgaagctctcctccgtcaccgcggccgatacggcagtgtactactgtgtgcgcgattacgacatcctcactggcgatgaggactactggggtcaaggcaccctagtcacggtgtcgtcgggaggtggtggatccgacatccagatgacacagactacatcctccctgtctgcctctctgggagacagagtcaccatcagttgcagggcaagtcaggacattagtaaatatttaaattggtatcagcagaaaccagatggaactgttaaactcctgatctaccatacatcaagattacactcaggagtcccatcaaggttcagtggcagtgggtctggaacagattattctctcaccattagcaacctggagcaagaagatattgccacttacttttgccaacagggtaatacgcttccgtacacgttcggaggggggaccaagctggagatcacaggtggcggtggctcgggcggtggtgggtcgggtggcggcggatctgaggtgaaactgcaggagtcaggacctggcctggtggcgccctcacagagcctgtccgtcacatgcactgtctcaggggtctcattacccgactatggtgtaagctggattcgccagcctccacgaaagggtctggagtggctgggagtaatatggggtagtgaaaccacatactataattcagctctcaaatccagactgaccatcatcaaggacaactccaagagccaagttttcttaaaaatgaacagtctgcaaactgacgacacagccatttactactgtgccaaacattattactacggtggtagctacgctatggactactggggccaaggaacctcagtcaccgtctcctctaa

SEQ ID NO: 33 - DNA, 1505 bp, Artificial Sequence
  affinity antibody mimetic
atggggtggagttgcatcattctgttcctcgtggcgaccgcaacaggcgtgcacagcgagatcgtgctcacccagtcaccagccaccttatccttaagtcccggcgaacgcgccaccctgtcctgcagagcgtcccagtcggtcagcagttatctggcgtggtaccagcagaagcccggccaagccccacgcctgctcatctacgacgcgtcgaatcgcgccacgggtattcccgcacggtttagcggctccggttcagggactgactttaccctgacgatctcgagtctagagccggaggacttcgcggtgtactactgccagcagtccagcaactggccgcgcaccttcggccagggcacaaaggtggagatcaaggggggcgggggctcgggtggcgggggctccggaggcgggggctcccaagtgtacctggttgaatcgggcgggggcgtggtgcagcctgggcgctcgctgcgcctcagttgcgccgcgtccggattcacattttccaactacgggatgcactgggtgcgccaagctccgggaaaggggctggagtgggtggccctgatctggtacgacggttccaataagtactatgccgatagcgtgaagggccggttcacgatatccagggataactccaagaacactctctatctgcagatgacctcactgcgcgtggaggacactgccgtctattactgcgcctccaatgtggatcactggggacagggcaccctggtgaccgtaagctcgggaggtggtggatccgacatccagatgacacagactacatcctccctgtctgcctctctgggagacagagtcaccatcagttgcagggcaagtcaggacattagtaaatatttaaattggtatcagcagaaaccagatggaactgttaaactcctgatctaccatacatcaagattacactcaggagtcccatcaaggttcagtggcagtgggtctggaacagattattctctcaccattagcaacctggagcaagaagatattgccacttacttttgccaacagggtaatacgcttccgtacacgttcggaggggggaccaagctggagatcacaggtggcggtggctcgggcggtggtgggtcgggtggcggcggatctgaggtgaaactgcaggagtcaggacctggcctggtggcgccctcacagagcctgtccgtcacatgcactgtctcaggggtctcattacccgactatggtgtaagctggattcgccagcctccacgaaagggtctggagtggctgggagtaatatggggtagtgaaaccacatactataattcagctctcaaatccagactgaccatcatcaaggacaactccaagagccaagttttcttaaaaatgaacagtctgcaaactgacgacacagccatttactactgtgccaaacattattactacggtggtagctacgctatggactactggggccaaggaacctcagtcaccgtctcctctaa

SEQ ID NO: 34 - DNA, 1497 bp, Artificial Sequence
  affinity antibody mimetic
atgggctggtcttgcatcatcctgtttctggtcgccaccgccaccggggtccacagtgagatcgttctcacccaatcccccgccacactgtcgctctccccaggcgagcgggccacgctgtcgtgtcgcgcgagccagagcgtttcctcctacctcgcctggtaccagcagaagccgggccaggcccctcgcctgctgatctacgatacttcgaatagagccaccggtatccctgcaaggttctccggatccgggtcagggacggatttcaccctgaccatttcctccctggagccagaggatttcgccgtgtactactgccagcagcgcagtaactggcctctgactttcggtggcggcacaaaggtggagatcaaggggggcggcggcagtgggggcgggggcagcgggggcggaggctcgcaggtccagctcgtggagtcggggggggacgtggtccagccaggcaggagcctgaggctgtcatgcgctgcgtccggcctgacgttcaccaactacggcttccactgggtgagacaggcacccgggaagggcctggaatgggtggccgtgatctggtacgacgggagcaagaagtactacgcagactcagtgaagggccgattcaccatcagccgggacaactctaagaacacactgtacctgcagatgaacaatttgcgcgccgaggataccgccgtatattattgcgccacaggcgacgactattggggacagggcaccctggtcacggtaagtagtggaggtggtggatccgatatccagctgacccaatcaccgtcgtccctgtctgcctccgtgggcgaccgggtgacgatcacctgtagtgcctcgagcagtgtacggttcatccactggtaccaacagaagcccggcaaggcaccaaagcggctgatctacgacaccagcaagctggcgtctggggtgcccagcaggttctcgggaagtggtagtggcacagacttcactctcaccatcagttcactccagccggaggactttgccacctactattgccagcagtggtcctcgtccccctttaccttcggccagggaacaaaggtggaaattaagggttcgacctccggggggggctccggtgggggctccggcggggggggctcatcggaggttcagctggtggagagcggcggcggcctggtgcagcccggcgggagtctgcggctgtcctgtgccgccagcggcttcaacatcaaggactactacattcactgggtgcggcaagccccaggcaagggtctggagtgggtggcttggattgaccctgaaaacggcgacactgagttcgtgccaaaattccaggggcgggcgaccatctccgccgacacctccaagaatacggcctacctgcagatgaactccctgcgcgccgaagacacagcggtctactactgcaagacagggggtttctggggccagggcaccctcgtgaccgtttcgagtgccgccggctaa

SEQ ID NO: 35 - DNA, 1521 bp, Artificial Sequence
  affinity antibody mimetic
atgggctggtcctgtatcatattattcctggtcgcgaccgccaccggggtgcactccgacatccagatgactcagtccccatcctccctgtcggcgtccgttggcgaccgggtctcgattacatgccgcgcctcccagggcatctcctcctggctcgcctggtaccagcagaagcctgagaaggcccccaagtcattaatctacgcagcctccaatctgaggtccggcgtgcccagtagattctcgggctccgggtcgggcactgattttaccctcaccatcagttcgctccagccagaggacttcgctacgtactattgccagcagtactattcctacccacgcaccttcgggcagggcaccaaggtcgagatcaagggcggcggcgggtccggcggaggcgggtctggcggtggtggttcgcagctgcagctgcaagagtccgggcctggcctcgtgaagcccagcgagaccctgtcattgacatgcaccgtgagtggggggagtctgtcccgctcctccttcttctggggctggattcgccagccgcccggcaaggggctggaatggatcgggtcgatctactacagtgggtcgacttactacaatccaagtctgaagagccgtgtgaccatctcagtggatacctcgaagaatcagttcagcctgaagctctcctccgtcaccgcggccgatacggcagtgtactactgtgtgcgcgattacgacatcctcactggcgatgaggactactggggtcaaggcaccctagtcacggtgtcgtcgggaggtggtggatccgatatccagctgacccaatcaccgtcgtccctgtctgcctccgtgggcgaccgggtgacgatcacctgtagtgcctcgagcagtgtacggttcatccactggtaccaacagaagcccggcaaggcaccaaagcggctgatctacgacaccagcaagctggcgtctggggtgcccagcaggttctcgggaagtggtagtggcacagacttcactctcaccatcagttcactccagccggaggactttgccacctactattgccagcagtggtcctcgtccccctttaccttcggccagggaacaaaggtggaaattaagggttcgacctccggggggggctccggtgggggctccggcggggggggctcatcggaggttcagctggtggagagcggcggcggcctggtgcagcccggcgggagtctgcggctgtcctgtgccgccagcggcttcaacatcaaggactactacattcactgggtgcggcaagccccaggcaagggtctggagtgggtggcttggattgaccctgaaaacggcgacactgagttcgtgccaaaattccaggggcgggcgaccatctccgccgacacctccaagaatacggcctacctgcagatgaactccctgcgcgccgaagacacagcggtctactactgcaagacagggggtttctggggccagggcaccctcgtgaccgtttcgagtgccgccggctaa

SEQ ID NO: 36 - DNA, 1497 bp, Artificial Sequence
  affinity antibody mimetic
atggggtggagttgcatcattctgttcctcgtggcgaccgcaacaggcgtgcacagcgagatcgtgctcacccagtcaccagccaccttatccttaagtcccggcgaacgcgccaccctgtcctgcagagcgtcccagtcggtcagcagttatctggcgtggtaccagcagaagcccggccaagccccacgcctgctcatctacgacgcgtcgaatcgcgccacgggtattcccgcacggtttagcggctccggttcagggactgactttaccctgacgatctcgagtctagagccggaggacttcgcggtgtactactgccagcagtccagcaactggccgcgcaccttcggccagggcacaaaggtggagatcaaggggggcgggggctcgggtggcgggggctccggaggcgggggctcccaagtgtacctggttgaatcgggcgggggcgtggtgcagcctgggcgctcgctgcgcctcagttgcgccgcgtccggattcacattttccaactacgggatgcactgggtgcgccaagctccgggaaaggggctggagtgggtggccctgatctggtacgacggttccaataagtactatgccgatagcgtgaagggccggttcacgatatccagggataactccaagaacactctctatctgcagatgacctcactgcgcgtggaggacactgccgtctattactgcgcctccaatgtggatcactggggacagggcaccctggtgaccgtaagctcgggaggtggtggatccgatatccagctgacccaatcaccgtcgtccctgtctgcctccgtgggcgaccgggtgacgatcacctgtagtgcctcgagcagtgtacggttcatccactggtaccaacagaagcccggcaaggcaccaaagcggctgatctacgacaccagcaagctggcgtctggggtgcccagcaggttctcgggaagtggtagtggcacagacttcactctcaccatcagttcactccagccggaggactttgccacctactattgccagcagtggtcctcgtccccctttaccttcggccagggaacaaaggtggaaattaagggttcgacctccggggggggctccggtgggggctccggcggggggggctcatcggaggttcagctggtggagagcggcggcggcctggtgcagcccggcgggagtctgcggctgtcctgtgccgccagcggcttcaacatcaaggactactacattcactgggtgcggcaagccccaggcaagggtctggagtgggtggcttggattgaccctgaaaacggcgacactgagttcgtgccaaaattccaggggcgggcgaccatctccgccgacacctccaagaatacggcctacctgcagatgaactccctgcgcgccgaagacacagcggtctactactgcaagacagggggtttctggggccagggcaccctcgtgaccgtttcgagtgccgccggctaa

SEQ ID NO: 37 - DNA, 1533 bp, Artificial Sequence
  affinity antibody mimetic
atgggttggagctgcatcattctgttcctcgtggcgacggctaccggggtgcactcggatatcgtgctgacccagtcgccggcaagcctcgccgtgtctctggggcagagagctacaatctcatgcaaagccagtcaaagtgtggattatgcgggggattcgtacatgaactggtatcagcagaagcccgggcagcctcccaagctgttgatctacgcggctagtaacctggagagcgggatcccagctcggttctccgggtccgggtccggaaccgacttcaccctcaacatccatccggtcgaggaggaggatgcggcaacctactactgccagcagtcgaatgaagatccgtacactttcggcgggggcaccaagctcgagataaagggaggaggcggctctggcgggggaggatctgggggcggcggctctcaggtccagctgcaacagtcaggccctgaactggtaaagcccggcgcttcggttaaaatctcgtgtaaggcttccgggtacgcgttctcctcctcctggatgaactgggtcaagcagcgcccaggaaagggcctggagtggattggccggatctatccgggcgatggcgacacaaactacaatggcaagttcaaggggaaggctactctcaccgcagataagtcctcgtctactgcttacatgcaacttagtagcctcacctcagaggattccgccgtgtatttctgcgcccgatccgattactatggcgattacggatttgcatattggggacaaggcaccctggttacggtcagcgccggaggtggtggatcccaggtacaactgcagcagtctgggcctgagctggagaagcctggcgcttcagtgaagatatcctgcaaggcttctggttactcattcactggctacaccatgaactgggtgaagcagagccatggaaagagccttgagtggattggacttattactccttacaatggtgcttctagctacaaccagaagttcaggggcaaggccacattaactgtagacaagtcatccagcacagcctacatggacctcctcagtctgacatctgaagactctgcagtctatttctgtgcaagggggggttacgacgggaggggttttgactactggggccaagggaccacggtcaccgtctcctcaggtggaggcggttcaggcggcggtggctctagcggtggcggatcggacatcgagctcactcagtctccagcaatcatgtctgcatctccaggggagaaggtcaccatgacctgcagtgccagctcaagtgtaagttacatgcactggtaccagcagaagtcaggcacctcccccaaaagatggatttacgacacatccaaactggcttctggagtcccaggtcgcttcagtggcagtgggtctggaaactcttactctctcacaatcagcagcgtggaggctgaagacgacgcaacttattactgccagcagtggagtaagcaccctctcacgtacggtgctgggacaaagttggaaatcaaataa

SEQ ID NO: 38 - DNA, 1533 bp, Artificial Sequence
  affinity antibody mimetic
atgggctggtcctgcatcatcctgttcctggtggctaccgccaccggtgttcactccgatatcgtcatgacccagtcgccagactcccttgctgtaagcctgggggagcgcgccaccatcaactgtaaagccagtcagtccgttgattacgccggcgagtcattcatgaactggtaccagcagaagcccggccagcctcctaagctactgatctacgccgcgtccaatctggagtcgggcgtcccagaccgcttttccggcagcgggtcgggtaccgatttcaccctgacgatctcctcgctccaggccgaggatgtggccgtgtattactgccagcagagtaacgaggatccatacaccttcggccagggaactaagctcgagatcaaagggggcggcggctccggcggcgggggctccggcggagggggcagtgaggtgcagctggtgcagtctggcgcagaggtgaagaaacccggagagtcgctcaagatctcgtgcaagggctcgggctacgccttttcgagttcgtggatgaactgggtgcgtcagatgcccggcaagggcctggagtggatgggccggatctatgcgggggatgcagataccgcgtactcgccgtcgtttcagggccaggttaccatcagcgcggacaaaagtatttccacggcgtacctgcagtggagttccctcaaggcgtccgacaccgccatgtactactgcgcccgcagtgactactatggggactacgggtttgcatactggggtcaggggaccctggtgaccgtgtcatcgggaggtggtggatcccaggtacaactgcagcagtctgggcctgagctggagaagcctggcgcttcagtgaagatatcctgcaaggcttctggttactcattcactggctacaccatgaactgggtgaagcagagccatggaaagagccttgagtggattggacttattactccttacaatggtgcttctagctacaaccagaagttcaggggcaaggccacattaactgtagacaagtcatccagcacagcctacatggacctcctcagtctgacatctgaagactctgcagtctatttctgtgcaagggggggttacgacgggaggggttttgactactggggccaagggaccacggtcaccgtctcctcaggtggaggcggttcaggcggcggtggctctagcggtggcggatcggacatcgagctcactcagtctccagcaatcatgtctgcatctccaggggagaaggtcaccatgacctgcagtgccagctcaagtgtaagttacatgcactggtaccagcagaagtcaggcacctcccccaaaagatggatttacgacacatccaaactggcttctggagtcccaggtcgcttcagtggcagtgggtctggaaactcttactctctcacaatcagcagcgtggaggctgaagacgacgcaacttattactgccagcagtggagtaagcaccctctcacgtacggtgctgggacaaagttggaaatcaaataa

SEQ ID NO: 39 - DNA, 1524 bp, Artificial Sequence
  affinity antibody mimetic
atgggctggtcctgcatcattctgttcctggtggccaccgccacgggggtgcactccgacattcagatgacccagtccccctcaagtctgtcagccagtgtgggcgaccgtgtgacaatcacctgcagggcctctaagtccgtgtccacttcggggtactcattcatgcactggtaccagcagaagcccggcaaagcacccaagctgctgatctacgtggggagccgcctggactatggcgtgccttcgcgcttttcgggcagcggatcgggcactgatttcactctgaccatctcctcactccaacccgaagacttcgcgacgtactactgccaacactcccgcgagctgccctggactttcggacagggcaccaaggttgagattaaaggcgggggcgggtcaggcgggggcggctccggcggcggaggaagtgaggtgcagctgctggagtcgggcggaggcctggtgcagcctggggggtcactccgactgagctgcgctgcatccgggttcaccttcagctcgtataccatgagctgggtgcgccaggcccccgggaagggcctggagtgggtgtctgtgatcgaccacgggggcgggtccacgcattatcccgatagcgtcaagggccggttcacgatctcgcgcgacaactctaagaatactctgtacctgcagatgaactccctgcgcgccgaagacactgcggtgtactattgtgccaggcaccgcggcaacccattcgactactggggccagggcaccctggtcacagtctcctccggaggtggtggatcccaggtacaactgcagcagtctgggcctgagctggagaagcctggcgcttcagtgaagatatcctgcaaggcttctggttactcattcactggctacaccatgaactgggtgaagcagagccatggaaagagccttgagtggattggacttattactccttacaatggtgcttctagctacaaccagaagttcaggggcaaggccacattaactgtagacaagtcatccagcacagcctacatggacctcctcagtctgacatctgaagactctgcagtctatttctgtgcaagggggggttacgacgggaggggttttgactactggggccaagggaccacggtcaccgtctcctcaggtggaggcggttcaggcggcggtggctctagcggtggcggatcggacatcgagctcactcagtctccagcaatcatgtctgcatctccaggggagaaggtcaccatgacctgcagtgccagctcaagtgtaagttacatgcactggtaccagcagaagtcaggcacctcccccaaaagatggatttacgacacatccaaactggcttctggagtcccaggtcgcttcagtggcagtgggtctggaaactcttactctctcacaatcagcagcgtggaggctgaagacgacgcaacttattactgccagcagtggagtaagcaccctctcacgtacggtgctgggacaaagttggaaatcaaataa

SEQ ID NO: 40 - DNA, 1545 bp, Artificial Sequence
  affinity antibody mimetic
atgggttggagctgcatcattctgttcctcgtggcgacggctaccggggtgcactcggatatcgtgctgacccagtcgccggcaagcctcgccgtgtctctggggcagagagctacaatctcatgcaaagccagtcaaagtgtggattatgcgggggattcgtacatgaactggtatcagcagaagcccgggcagcctcccaagctgttgatctacgcggctagtaacctggagagcgggatcccagctcggttctccgggtccgggtccggaaccgacttcaccctcaacatccatccggtcgaggaggaggatgcggcaacctactactgccagcagtcgaatgaagatccgtacactttcggcgggggcaccaagctcgagataaagggaggaggcggctctggcgggggaggatctgggggcggcggctctcaggtccagctgcaacagtcaggccctgaactggtaaagcccggcgcttcggttaaaatctcgtgtaaggcttccgggtacgcgttctcctcctcctggatgaactgggtcaagcagcgcccaggaaagggcctggagtggattggccggatctatccgggcgatggcgacacaaactacaatggcaagttcaaggggaaggctactctcaccgcagataagtcctcgtctactgcttacatgcaacttagtagcctcacctcagaggattccgccgtgtatttctgcgcccgatccgattactatggcgattacggatttgcatattggggacaaggcaccctggttacggtcagcgccggaggtggtggatccgacatccagatgacccagtccccttcctccctctctgcctctgtgggagaccgcgttaccatcacatgccgagcttcccaggacgtgaacacagccgtggcctggtaccagcagaagcccgggaaggcacccaaactcctcatctactccgcctccttcctatacagtggcgtgccttcccgattctccggctccaggagtggcacggactttacgctcaccattagtagcctgcagcccgaagacttcgcgacctactattgtcagcaacactacacgacgccaccaactttcggccagggtaccaaggtcgagattaagcgaaccggcagtaccagtgggtctggcaagcccggcagcggcgagggatccgaggtccagctggtcgagtccggcgggggcctggtgcagccgggcggctcgctgaggttatcttgcgccgccagtggcttcaacatcaaggatacttacatccactgggtgaggcaggctccgggcaagggcctggaatgggtggctaggatctaccctactaacgggtacacacgctacgcagattcggtgaaaggccgcttcactatctccgccgacacctcgaagaacactgcttacctgcagatgaactccctcagggccgaagatactgcagtctactactgctcccgctggggtggggacggcttctacgccatggacgtgtggggtcagggcactctagttacagtgtcatcctaa

SEQ ID NO: 41 - DNA, 1545 bp, Artificial Sequence
  affinity antibody mimetic
atgggctggtcctgcatcatcctgttcctggtggctaccgccaccggtgttcactccgatatcgtcatgacccagtcgccagactcccttgctgtaagcctgggggagcgcgccaccatcaactgtaaagccagtcagtccgttgattacgccggcgagtcattcatgaactggtaccagcagaagcccggccagcctcctaagctactgatctacgccgcgtccaatctggagtcgggcgtcccagaccgcttttccggcagcgggtcgggtaccgatttcaccctgacgatctcctcgctccaggccgaggatgtggccgtgtattactgccagcagagtaacgaggatccatacaccttcggccagggaactaagctcgagatcaaagggggcggcggctccggcggcgggggctccggcggagggggcagtgaggtgcagctggtgcagtctggcgcagaggtgaagaaacccggagagtcgctcaagatctcgtgcaagggctcgggctacgccttttcgagttcgtggatgaactgggtgcgtcagatgcccggcaagggcctggagtggatgggccggatctatgcgggggatgcagataccgcgtactcgccgtcgtttcagggccaggttaccatcagcgcggacaaaagtatttccacggcgtacctgcagtggagttccctcaaggcgtccgacaccgccatgtactactgcgcccgcagtgactactatggggactacgggtttgcatactggggtcaggggaccctggtgaccgtgtcatcgggaggtggtggatccgacatccagatgacccagtccccttcctccctctctgcctctgtgggagaccgcgttaccatcacatgccgagcttcccaggacgtgaacacagccgtggcctggtaccagcagaagcccgggaaggcacccaaactcctcatctactccgcctccttcctatacagtggcgtgccttcccgattctccggctccaggagtggcacggactttacgctcaccattagtagcctgcagcccgaagacttcgcgacctactattgtcagcaacactacacgacgccaccaactttcggccagggtaccaaggtcgagattaagcgaaccggcagtaccagtgggtctggcaagcccggcagcggcgagggatccgaggtccagctggtcgagtccggcgggggcctggtgcagccgggcggctcgctgaggttatcttgcgccgccagtggcttcaacatcaaggatacttacatccactgggtgaggcaggctccgggcaagggcctggaatgggtggctaggatctaccctactaacgggtacacacgctacgcagattcggtgaaaggccgcttcactatctccgccgacacctcgaagaacactgcttacctgcagatgaactccctcagggccgaagatactgcagtctactactgctcccgctggggtggggacggcttctacgccatggacgtgtggggtcagggcactctagttacagtgtcatcctaa

SEQ ID NO: 42 - DNA, 1536 bp, Artificial Sequence
  affinity antibody mimetic
atgggctggtcctgcatcattctgttcctggtggccaccgccacgggggtgcactccgacattcagatgacccagtccccctcaagtctgtcagccagtgtgggcgaccgtgtgacaatcacctgcagggcctctaagtccgtgtccacttcggggtactcattcatgcactggtaccagcagaagcccggcaaagcacccaagctgctgatctacgtggggagccgcctggactatggcgtgccttcgcgcttttcgggcagcggatcgggcactgatttcactctgaccatctcctcactccaacccgaagacttcgcgacgtactactgccaacactcccgcgagctgccctggactttcggacagggcaccaaggttgagattaaaggcgggggcgggtcaggcgggggcggctccggcggcggaggaagtgaggtgcagctgctggagtcgggcggaggcctggtgcagcctggggggtcactccgactgagctgcgctgcatccgggttcaccttcagctcgtataccatgagctgggtgcgccaggcccccgggaagggcctggagtgggtgtctgtgatcgaccacgggggcgggtccacgcattatcccgatagcgtcaagggccggttcacgatctcgcgcgacaactctaagaatactctgtacctgcagatgaactccctgcgcgccgaagacactgcggtgtactattgtgccaggcaccgcggcaacccattcgactactggggccagggcaccctggtcacagtctcctccggaggtggtggatccgacatccagatgacccagtccccttcctccctctctgcctctgtgggagaccgcgttaccatcacatgccgagcttcccaggacgtgaacacagccgtggcctggtaccagcagaagcccgggaaggcacccaaactcctcatctactccgcctccttcctatacagtggcgtgccttcccgattctccggctccaggagtggcacggactttacgctcaccattagtagcctgcagcccgaagacttcgcgacctactattgtcagcaacactacacgacgccaccaactttcggccagggtaccaaggtcgagattaagcgaaccggcagtaccagtgggtctggcaagcccggcagcggcgagggatccgaggtccagctggtcgagtccggcgggggcctggtgcagccgggcggctcgctgaggttatcttgcgccgccagtggcttcaacatcaaggatacttacatccactgggtgaggcaggctccgggcaagggcctggaatgggtggctaggatctaccctactaacgggtacacacgctacgcagattcggtgaaaggccgcttcactatctccgccgacacctcgaagaacactgcttacctgcagatgaactccctcagggccgaagatactgcagtctactactgctcccgctggggtggggacggcttctacgccatggacgtgtggggtcagggcactctagttacagtgtcatcctaa

SEQ ID NO: 43 - DNA, 1467 bp, Artificial Sequence
  affinity antibody mimetic
atgggttggagctgcatcattctgttcctcgtggcgacggctaccggggtgcactcggatatcgtgctgacccagtcgccggcaagcctcgccgtgtctctggggcagagagctacaatctcatgcaaagccagtcaaagtgtggattatgcgggggattcgtacatgaactggtatcagcagaagcccgggcagcctcccaagctgttgatctacgcggctagtaacctggagagcgggatcccagctcggttctccgggtccgggtccggaaccgacttcaccctcaacatccatccggtcgaggaggaggatgcggcaacctactactgccagcagtcgaatgaagatccgtacactttcggcgggggcaccaagctcgagataaagggaggaggcggctctggcgggggaggatctgggggcggcggctctcaggtccagctgcaacagtcaggccctgaactggtaaagcccggcgcttcggttaaaatctcgtgtaaggcttccgggtacgcgttctcctcctcctggatgaactgggtcaagcagcgcccaggaaagggcctggagtggattggccggatctatccgggcgatggcgacacaaactacaatggcaagttcaaggggaaggctactctcaccgcagataagtcctcgtctactgcttacatgcaacttagtagcctcacctcagaggattccgccgtgtatttctgcgcccgatccgattactatggcgattacggatttgcatattggggacaaggcaccctggttacggtcagcgccaccacgacgccagcgccgcgaccaccaacaccggcgcccaccatcgcgtcgcagcccctgtccctgcgcccagaggcgtgccggccagcggcggggggcgcagtgcacacgagggggctggacttcgcctgtgatatctacatctgggcgcccttggccgggacttgtggggtccttctcctgtcactggttatcaccctttactgcaaacggggcagaaagaaactcctgtatatattcaaacaaccatttatgagaccagtacaaactactcaagaggaagatggctgtagctgccgatttccagaagaagaagaaggaggatgtgaactgagagtgaagttcagcaggagcgcagacgcccccgcgtacaagcagggccagaaccagctctataacgagctcaatctaggacgaagagaggagtacgacgttttggacaagagacgtggccgggaccctgagatggggggaaagccgagaaggaagaaccctcaggaaggcctgtacaatgaactgcagaaagataagatggcggaggcctacagtgagattgggatgaaaggcgagcgccggaggggcaaggggcacgatggcctttaccagggtctcagtacagccaccaaggacacctacgacgcccttcacatgcaggccctgccccctcgctaa

SEQ ID NO: 44 - DNA, 1467 bp, Artificial Sequence
  affinity antibody mimetic
atgggctggtcctgcatcatcctgttcctggtggctaccgccaccggtgttcactccgatatcgtcatgacccagtcgccagactcccttgctgtaagcctgggggagcgcgccaccatcaactgtaaagccagtcagtccgttgattacgccggcgagtcattcatgaactggtaccagcagaagcccggccagcctcctaagctactgatctacgccgcgtccaatctggagtcgggcgtcccagaccgcttttccggcagcgggtcgggtaccgatttcaccctgacgatctcctcgctccaggccgaggatgtggccgtgtattactgccagcagagtaacgaggatccatacaccttcggccagggaactaagctcgagatcaaagggggcggcggctccggcggcgggggctccggcggagggggcagtgaggtgcagctggtgcagtctggcgcagaggtgaagaaacccggagagtcgctcaagatctcgtgcaagggctcgggctacgccttttcgagttcgtggatgaactgggtgcgtcagatgcccggcaagggcctggagtggatgggccggatctatgcgggggatgcagataccgcgtactcgccgtcgtttcagggccaggttaccatcagcgcggacaaaagtatttccacggcgtacctgcagtggagttccctcaaggcgtccgacaccgccatgtactactgcgcccgcagtgactactatggggactacgggtttgcatactggggtcaggggaccctggtgaccgtgtcatcgaccacgacgccagcgccgcgaccaccaacaccggcgcccaccatcgcgtcgcagcccctgtccctgcgcccagaggcgtgccggccagcggcggggggcgcagtgcacacgagggggctggacttcgcctgtgatatctacatctgggcgcccttggccgggacttgtggggtccttctcctgtcactggttatcaccctttactgcaaacggggcagaaagaaactcctgtatatattcaaacaaccatttatgagaccagtacaaactactcaagaggaagatggctgtagctgccgatttccagaagaagaagaaggaggatgtgaactgagagtgaagttcagcaggagcgcagacgcccccgcgtacaagcagggccagaaccagctctataacgagctcaatctaggacgaagagaggagtacgacgttttggacaagagacgtggccgggaccctgagatggggggaaagccgagaaggaagaaccctcaggaaggcctgtacaatgaactgcagaaagataagatggcggaggcctacagtgagattgggatgaaaggcgagcgccggaggggcaaggggcacgatggcctttaccagggtctcagtacagccaccaaggacacctacgacgcccttcacatgcaggccctgccccctcgctaa

SEQ ID NO: 45 - DNA, 1458 bp, Artificial Sequence
  affinity antibody mimetic
atgggctggtcctgcatcattctgttcctggtggccaccgccacgggggtgcactccgacattcagatgacccagtccccctcaagtctgtcagccagtgtgggcgaccgtgtgacaatcacctgcagggcctctaagtccgtgtccacttcggggtactcattcatgcactggtaccagcagaagcccggcaaagcacccaagctgctgatctacgtggggagccgcctggactatggcgtgccttcgcgcttttcgggcagcggatcgggcactgatttcactctgaccatctcctcactccaacccgaagacttcgcgacgtactactgccaacactcccgcgagctgccctggactttcggacagggcaccaaggttgagattaaaggcgggggcgggtcaggcgggggcggctccggcggcggaggaagtgaggtgcagctgctggagtcgggcggaggcctggtgcagcctggggggtcactccgactgagctgcgctgcatccgggttcaccttcagctcgtataccatgagctgggtgcgccaggcccccgggaagggcctggagtgggtgtctgtgatcgaccacgggggcgggtccacgcattatcccgatagcgtcaagggccggttcacgatctcgcgcgacaactctaagaatactctgtacctgcagatgaactccctgcgcgccgaagacactgcggtgtactattgtgccaggcaccgcggcaacccattcgactactggggccagggcaccctggtcacagtctcctccaccacgacgccagcgccgcgaccaccaacaccggcgcccaccatcgcgtcgcagcccctgtccctgcgcccagaggcgtgccggccagcggcggggggcgcagtgcacacgagggggctggacttcgcctgtgatatctacatctgggcgcccttggccgggacttgtggggtccttctcctgtcactggttatcaccctttactgcaaacggggcagaaagaaactcctgtatatattcaaacaaccatttatgagaccagtacaaactactcaagaggaagatggctgtagctgccgatttccagaagaagaagaaggaggatgtgaactgagagtgaagttcagcaggagcgcagacgcccccgcgtacaagcagggccagaaccagctctataacgagctcaatctaggacgaagagaggagtacgacgttttggacaagagacgtggccgggaccctgagatggggggaaagccgagaaggaagaaccctcaggaaggcctgtacaatgaactgcagaaagataagatggcggaggcctacagtgagattgggatgaaaggcgagcgccggaggggcaaggggcacgatggcctttaccagggtctcagtacagccaccaaggacacctacgacgcccttcacatgcaggccctgccccctcgctaa

SEQ ID NO: 46 - DNA, 1538 bp, Artificial Sequence
  affinity antibody mimetic
atgggttggagctgcatcattctgttcctcgtggcgacggctaccggggtgcactcggatatcgtgctgacccagtcgccggcaagcctcgccgtgtctctggggcagagagctacaatctcatgcaaagccagtcaaagtgtggattatgcgggggattcgtacatgaactggtatcagcagaagcccgggcagcctcccaagctgttgatctacgcggctagtaacctggagagcgggatcccagctcggttctccgggtccgggtccggaaccgacttcaccctcaacatccatccggtcgaggaggaggatgcggcaacctactactgccagcagtcgaatgaagatccgtacactttcggcgggggcaccaagctcgagataaagggaggaggcggctctggcgggggaggatctgggggcggcggctctcaggtccagctgcaacagtcaggccctgaactggtaaagcccggcgcttcggttaaaatctcgtgtaaggcttccgggtacgcgttctcctcctcctggatgaactgggtcaagcagcgcccaggaaagggcctggagtggattggccggatctatccgggcgatggcgacacaaactacaatggcaagttcaaggggaaggctactctcaccgcagataagtcctcgtctactgcttacatgcaacttagtagcctcacctcagaggattccgccgtgtatttctgcgcccgatccgattactatggcgattacggatttgcatattggggacaaggcaccctggttacggtcagcgccggaggtggtggatccgacatccagatgacacagactacatcctccctgtctgcctctctgggagacagagtcaccatcagttgcagggcaagtcaggacattagtaaatatttaaattggtatcagcagaaaccagatggaactgttaaactcctgatctaccatacatcaagattacactcaggagtcccatcaaggttcagtggcagtgggtctggaacagattattctctcaccattagcaacctggagcaagaagatattgccacttacttttgccaacagggtaatacgcttccgtacacgttcggaggggggaccaagctggagatcacaggtggcggtggctcgggcggtggtgggtcgggtggcggcggatctgaggtgaaactgcaggagtcaggacctggcctggtggcgccctcacagagcctgtccgtcacatgcactgtctcaggggtctcattacccgactatggtgtaagctggattcgccagcctccacgaaagggtctggagtggctgggagtaatatggggtagtgaaaccacatactataattcagctctcaaatccagactgaccatcatcaaggacaactccaagagccaagttttcttaaaaatgaacagtctgcaaactgacgacacagccatttactactgtgccaaacattattactacggtggtagctacgctatggactactggggccaaggaacctcagtcaccgtctcctctaa

SEQ ID NO: 47 - DNA, 1538 bp, Artificial Sequence
  affinity antibody mimetic
atgggctggtcctgcatcatcctgttcctggtggctaccgccaccggtgttcactccgatatcgtcatgacccagtcgccagactcccttgctgtaagcctgggggagcgcgccaccatcaactgtaaagccagtcagtccgttgattacgccggcgagtcattcatgaactggtaccagcagaagcccggccagcctcctaagctactgatctacgccgcgtccaatctggagtcgggcgtcccagaccgcttttccggcagcgggtcgggtaccgatttcaccctgacgatctcctcgctccaggccgaggatgtggccgtgtattactgccagcagagtaacgaggatccatacaccttcggccagggaactaagctcgagatcaaagggggcggcggctccggcggcgggggctccggcggagggggcagtgaggtgcagctggtgcagtctggcgcagaggtgaagaaacccggagagtcgctcaagatctcgtgcaagggctcgggctacgccttttcgagttcgtggatgaactgggtgcgtcagatgcccggcaagggcctggagtggatgggccggatctatgcgggggatgcagataccgcgtactcgccgtcgtttcagggccaggttaccatcagcgcggacaaaagtatttccacggcgtacctgcagtggagttccctcaaggcgtccgacaccgccatgtactactgcgcccgcagtgactactatggggactacgggtttgcatactggggtcaggggaccctggtgaccgtgtcatcgggaggtggtggatccgacatccagatgacacagactacatcctccctgtctgcctctctgggagacagagtcaccatcagttgcagggcaagtcaggacattagtaaatatttaaattggtatcagcagaaaccagatggaactgttaaactcctgatctaccatacatcaagattacactcaggagtcccatcaaggttcagtggcagtgggtctggaacagattattctctcaccattagcaacctggagcaagaagatattgccacttacttttgccaacagggtaatacgcttccgtacacgttcggaggggggaccaagctggagatcacaggtggcggtggctcgggcggtggtgggtcgggtggcggcggatctgaggtgaaactgcaggagtcaggacctggcctggtggcgccctcacagagcctgtccgtcacatgcactgtctcaggggtctcattacccgactatggtgtaagctggattcgccagcctccacgaaagggtctggagtggctgggagtaatatggggtagtgaaaccacatactataattcagctctcaaatccagactgaccatcatcaaggacaactccaagagccaagttttcttaaaaatgaacagtctgcaaactgacgacacagccatttactactgtgccaaacattattactacggtggtagctacgctatggactactggggccaaggaacctcagtcaccgtctcctctaa

SEQ ID NO: 48 - DNA, 1529 bp, Artificial Sequence
  affinity antibody mimetic
atgggctggtcctgcatcattctgttcctggtggccaccgccacgggggtgcactccgacattcagatgacccagtccccctcaagtctgtcagccagtgtgggcgaccgtgtgacaatcacctgcagggcctctaagtccgtgtccacttcggggtactcattcatgcactggtaccagcagaagcccggcaaagcacccaagctgctgatctacgtggggagccgcctggactatggcgtgccttcgcgcttttcgggcagcggatcgggcactgatttcactctgaccatctcctcactccaacccgaagacttcgcgacgtactactgccaacactcccgcgagctgccctggactttcggacagggcaccaaggttgagattaaaggcgggggcgggtcaggcgggggcggctccggcggcggaggaagtgaggtgcagctgctggagtcgggcggaggcctggtgcagcctggggggtcactccgactgagctgcgctgcatccgggttcaccttcagctcgtataccatgagctgggtgcgccaggcccccgggaagggcctggagtgggtgtctgtgatcgaccacgggggcgggtccacgcattatcccgatagcgtcaagggccggttcacgatctcgcgcgacaactctaagaatactctgtacctgcagatgaactccctgcgcgccgaagacactgcggtgtactattgtgccaggcaccgcggcaacccattcgactactggggccagggcaccctggtcacagtctcctccggaggtggtggatccgacatccagatgacacagactacatcctccctgtctgcctctctgggagacagagtcaccatcagttgcagggcaagtcaggacattagtaaatatttaaattggtatcagcagaaaccagatggaactgttaaactcctgatctaccatacatcaagattacactcaggagtcccatcaaggttcagtggcagtgggtctggaacagattattctctcaccattagcaacctggagcaagaagatattgccacttacttttgccaacagggtaatacgcttccgtacacgttcggaggggggaccaagctggagatcacaggtggcggtggctcgggcggtggtgggtcgggtggcggcggatctgaggtgaaactgcaggagtcaggacctggcctggtggcgccctcacagagcctgtccgtcacatgcactgtctcaggggtctcattacccgactatggtgtaagctggattcgccagcctccacgaaagggtctggagtggctgggagtaatatggggtagtgaaaccacatactataattcagctctcaaatccagactgaccatcatcaaggacaactccaagagccaagttttcttaaaaatgaacagtctgcaaactgacgacacagccatttactactgtgccaaacattattactacggtggtagctacgctatggactactggggccaaggaacctcagtcaccgtctcctctaa

SEQ ID NO: 49 - DNA, 1029 bp, Artificial Sequence
  affinity antibody mimetic
atgcagatcccacaggcgccctggccagtcgtctgggcggtgctacaactgggctggcggccaggatggttcttagactccccagacaggccctggaacccccccaccttctccccagccctgctcgtggtgaccgaaggggacaacgccaccttcacctgcagcttctccaacacatcggagagcttcgtgctaaactggtaccgcatgagccccagcaaccagacggacaagctggccgccttccccgaggaccgcagccagcccggccaggactgccgcttccgtgtcacacaactgcccaacgggcgtgacttccacatgagcgtggtcagggcccggcgcaatgacagcggcacctacctctgtggggccatctccctggcccccaaggcgcagatcaaagagagcctgcgggcagagctcagggtgacagagagaagggcagaagtgcccacagcccaccccagcccctcacccaggccagccggccagttccaaaccctggtgttttgggtgctggtggtggttggtggagtcctggcttgctatagcttgctagtaacagtggcctttattattttctgggtgctttactgcaaccacaggaaccgaagacgtgtttgcaaatgtccccggcctgtggtcaaatcgggagacaagcccagcctttcggcgagatacgtcctgagagtgaagttcagcaggagcgcagacgcccccgcgtacaagcagggccagaaccagctctataacgagctcaatctaggacgaagagaggagtacgacgttttggacaagagacgtggccgggaccctgagatggggggaaagccgagaaggaagaaccctcaggaaggcctgtacaatgaactgcagaaagataagatggcggaggcctacagtgagattgggatgaaaggcgagcgccggaggggcaaggggcacgatggcctttaccagggtctcagtacagccaccaaggacacctacgacgcccttcacatgcaggccctgccccctcgctaa

SEQ ID NO: 50 - DNA, 1053 bp, Artificial Sequence
  affinity antibody mimetic
atgcagatcccacaggcgccctggccagtcgtctgggcggtgctacaactgggctggcggccaggatggttcttagactccccagacaggccctggaacccccccaccttctccccagccctgctcgtggtgaccgaaggggacaacgccaccttcacctgcagcttctccaacacatcggagagcttcgtgctaaactggtaccgcatgagccccagcaaccagacggacaagctggccgccttccccgaggaccgcagccagcccggccaggactgccgcttccgtgtcacacaactgcccaacgggcgtgacttccacatgagcgtggtcagggcccggcgcaatgacagcggcacctacctctgtggggccatctccctggcccccaaggcgcagatcaaagagagcctgcgggcagagctcagggtgacagagagaagggcagaagtgcccacagcccaccccagcccctcacccaggccagccggccagttccaaaccctggtgttttgggtgctggtggtggttggtggagtcctggcttgctatagcttgctagtaacagtggcctttattattttctgggtgtgtgtcaggtgccggcaccgaaggcgccaagcagagcggatgtctcagatcaagagactcctcagtgagaagaagacctgccagtgccctcaccggtttcagaagacatgtagccccattctgagagtgaagttcagcaggagcgcagacgcccccgcgtacaagcagggccagaaccagctctataacgagctcaatctaggacgaagagaggagtacgacgttttggacaagagacgtggccgggaccctgagatggggggaaagccgagaaggaagaaccctcaggaaggcctgtacaatgaactgcagaaagataagatggcggaggcctacagtgagattgggatgaaaggcgagcgccggaggggcaaggggcacgatggcctttaccagggtctcagtacagccaccaaggacacctacgacgcccttcacatgcaggccctgccccctcgctaa

SEQ ID NO: 51 - DNA, 1056 bp, Artificial Sequence
  affinity antibody mimetic
atgcagatcccacaggcgccctggccagtcgtctgggcggtgctacaactgggctggcggccaggatggttcttagactccccagacaggccctggaacccccccaccttctccccagccctgctcgtggtgaccgaaggggacaacgccaccttcacctgcagcttctccaacacatcggagagcttcgtgctaaactggtaccgcatgagccccagcaaccagacggacaagctggccgccttccccgaggaccgcagccagcccggccaggactgccgcttccgtgtcacacaactgcccaacgggcgtgacttccacatgagcgtggtcagggcccggcgcaatgacagcggcacctacctctgtggggccatctccctggcccccaaggcgcagatcaaagagagcctgcgggcagagctcagggtgacagagagaagggcagaagtgcccacagcccaccccagcccctcacccaggccagccggccagttccaaaccctggtgttttgggtgctggtggtggttggtggagtcctggcttgctatagcttgctagtaacagtggcctttattattttctgggtgaggagtaagaggagcaggctcctgcacagtgactacatgaacatgactccccgccgccccgggcccacccgcaagcattaccagccctatgccccaccacgcgacttcgcagcctatcgctccgatagagtgaagttcagcaggagcgcagacgcccccgcgtaccagcagggccagaaccagctctataacgagctcaatctaggacgaagagaggagtacgatgttttggacaagagacgtggccgggaccctgagatggggggaaagccgagaaggaagaaccctcaggaaggcctgtacaatgaactgcagaaagataagatggcggaggcctacagtgagattgggatgaaaggcgagcgccggaggggcaaggggcacgatggcctttaccagggtctcagtacagccaccaaggacacctacgacgcccttcacatgcaggccctgccccctcgctaa

SEQ ID NO: 52 - DNA, 1053 bp, Artificial Sequence
  affinity antibody mimetic
atgcagatcccacaggcgccctggccagtcgtctgggcggtgctacaactgggctggcggccaggatggttcttagactccccagacaggccctggaacccccccaccttctccccagccctgctcgtggtgaccgaaggggacaacgccaccttcacctgcagcttctccaacacatcggagagcttcgtgctaaactggtaccgcatgagccccagcaaccagacggacaagctggccgccttccccgaggaccgcagccagcccggccaggactgccgcttccgtgtcacacaactgcccaacgggcgtgacttccacatgagcgtggtcagggcccggcgcaatgacagcggcacctacctctgtggggccatctccctggcccccaaggcgcagatcaaagagagcctgcgggcagagctcagggtgacagagagaagggcagaagtgcccacagcccaccccagcccctcacccaggccagccggccagttccaaaccctggtgttttgggtgctggtggtggttggtggagtcctggcttgctatagcttgctagtaacagtggcctttattattttctgggtgcggggcagaaagaaactcctgtatatattcaaacaaccatttatgagaccagtacaaactactcaagaggaagatggctgtagctgccgatttccagaagaagaagaaggaggatgtgaagatagagtgaagttcagcaggagcgcagacgcccccgcgtaccagcagggccagaaccagctctataacgagctcaatctaggacgaagagaggagtacgatgttttggacaagagacgtggccgggaccctgagatggggggaaagccgagaaggaagaaccctcaggaaggcctgtacaatgaactgcagaaagataagatggcggaggcctacagtgagattgggatgaaaggcgagcgccggaggggcaaggggcacgatggcctttaccagggtctcagtacagccaccaaggacacctacgacgcccttcacatgcaggccctgccccctcgctaa